European Patent Application EP 4 755 917 A1, published June 10, 2026. Title: INNOVENT BIOLOGICS (SUZHOU) CO., LTD. Applicant: INNOVENT BIOLOGICS (SUZHOU) CO., LTD. The sequence listing filed with the application follows.

SEQUENCE LISTING (30 sequences)

SEQ ID NO: 1 - protein, 10 aa, synthetic construct
GYSFTGYRIH

SEQ ID NO: 2 - protein, 17 aa, synthetic construct
YVDPYDDKTDYSQKSKG

SEQ ID NO: 3 - protein, 5 aa, synthetic construct
EGFAY

SEQ ID NO: 4 - protein, 114 aa, synthetic construct
EVQLVQSGAEVKKPGATVKISCKVSGYSFTGYRIHWVQQAPGKGLEWMGYVDPYDDKTDYSQKSKGRVTITADTSTDTAYMELSSLRSEDTAVYYCAREGFAYWGQGTLVTVSS

SEQ ID NO: 5 - protein, 10 aa, synthetic construct
TSSSSLRYMH

SEQ ID NO: 6 - protein, 7 aa, synthetic construct
NTFDLAS

SEQ ID NO: 7 - protein, 9 aa, synthetic construct
QQRTTYPPT

SEQ ID NO: 8 - protein, 106 aa, synthetic construct
DIQMTQSPSSLSASVGDRVTITCTSSSSLRYMHWYQQKPGKAPKLLIYNTFDLASGVPSRFSGSGSGTDFTLTISSLQPEDFATYYCQQRTTYPPTFGQGTKLEIK

SEQ ID NO: 9 - protein, 441 aa, synthetic construct
EVQLVQSGAEVKKPGATVKISCKVSGYSFTGYRIHWVQQAPGKGLEWMGYVDPYDDKTDYSQKSKGRVTITADTSTDTAYMELSSLRSEDTAVYYCAREGFAYWGQGTLVTVSSASTKGPSVFPLAPCSRSTSESTAALGCLVKDYFPEPVTVSWNSGALTSGVHTFPAVLQSSGLYSLSSVVTVPSSSLGTKTYTCNVDHKPSNTKVDKRVESKYGPPCPPCPAPEFLGGPSVFLFPPKPKDTLMISRTPEVTCVVVDVSQEDPEVQFNWYVDGVEVHNAKTKPREEQFNSTYRVVSVLTVLHQDWLNGKEYKCKVSNKGLPSSIEKTISKAKGQPREPQVYTLPPSQEEMTKNQVSLTCLVKGFYPSDIAVEWESNGQPENNYKTTPPVLDSDGSFFLYSRLTVDKSRWQEGNVFSCSVMHEALHNHYTQKSLSLSLGK

SEQ ID NO: 10 - protein, 213 aa, synthetic construct
DIQMTQSPSSLSASVGDRVTITCTSSSSLRYMHWYQQKPGKAPKLLIYNTFDLASGVPSRFSGSGSGTDFTLTISSLQPEDFATYYCQQRTTYPPTFGQGTKLEIKRTVAAPSVFIFPPSDEQLKSGTASVVCLLNNFYPREAKVQWKVDNALQSGNSQESVTEQDSKDSTYSLSSTLTLSKADYEKHKVYACEVTHQGLSSPVTKSFNRGEC

SEQ ID NO: 11 - protein, 11 aa, synthetic construct
GYAVTGDYAWS

SEQ ID NO: 12 - protein, 16 aa, synthetic construct
YISSSAGTNYNPSLKS

SEQ ID NO: 13 - protein, 14 aa, synthetic construct
DLYYGGRNQWYFDV

SEQ ID NO: 14 - protein, 123 aa, synthetic construct
QVQLQESGPGLVKPSQTLSLTCTVSGYAVTGDYAWSWIRQPPGKRLEWIGYISSSAGTNYNPSLKSRVTISVDTSKNQFSLKLSSVTAADTAVYYCARDLYYGGRNQWYFDVWGQGTLVTVSS

SEQ ID NO: 15 - protein, 10 aa, synthetic construct
SATSSIIYMH

SEQ ID NO: 16 - protein, 7 aa, synthetic construct
DTSKLPS

SEQ ID NO: 17 - protein, 9 aa, synthetic construct
HQRSSFPFT

SEQ ID NO: 18 - protein, 106 aa, synthetic construct
DIQMTQSPSSLSASVGDRVTITCSATSSIIYMHWYQQKPGKAPKLLIYDTSKLPSGVPSRFSGSGSGTDFTLTISSLQPEDFATYYCHQRSSFPFTFGGGTKVEIK

SEQ ID NO: 19 - protein, 450 aa, synthetic construct
QVQLQESGPGLVKPSQTLSLTCTVSGYAVTGDYAWSWIRQPPGKRLEWIGYISSSAGTNYNPSLKSRVTISVDTSKNQFSLKLSSVTAADTAVYYCARDLYYGGRNQWYFDVWGQGTLVTVSSASTKGPSVFPLAPCSRSTSESTAALGCLVKDYFPEPVTVSWNSGALTSGVHTFPAVLQSSGLYSLSSVVTVPSSSLGTKTYTCNVDHKPSNTKVDKRVESKYGPPCPPCPAPEFLGGPSVFLFPPKPKDTLMISRTPEVTCVVVDVSQEDPEVQFNWYVDGVEVHNAKTKPREEQFNSTYRVVSVLTVLHQDWLNGKEYKCKVSNKGLPSSIEKTISKAKGQPREPQVYTLPPSQEEMTKNQVSLTCLVKGFYPSDIAVEWESNGQPENNYKTTPPVLDSDGSFFLYSRLTVDKSRWQEGNVFSCSVMHEALHNHYTQKSLSLSLGK

SEQ ID NO: 20 - protein, 213 aa, synthetic construct
DIQMTQSPSSLSASVGDRVTITCSATSSIIYMHWYQQKPGKAPKLLIYDTSKLPSGVPSRFSGSGSGTDFTLTISSLQPEDFATYYCHQRSSFPFTFGGGTKVEIKRTVAAPSVFIFPPSDEQLKSGTASVVCLLNNFYPREAKVQWKVDNALQSGNSQESVTEQDSKDSTYSLSSTLTLSKADYEKHKVYACEVTHQGLSSPVTKSFNRGEC

SEQ ID NO: 21 - protein, 327 aa, synthetic construct
ASTKGPSVFPLAPCSRSTSESTAALGCLVKDYFPEPVTVSWNSGALTSGVHTFPAVLQSSGLYSLSSVVTVPSSSLGTKTYTCNVDHKPSNTKVDKRVESKYGPPCPPCPAPEFLGGPSVFLFPPKPKDTLMISRTPEVTCVVVDVSQEDPEVQFNWYVDGVEVHNAKTKPREEQFNSTYRVVSVLTVLHQDWLNGKEYKCKVSNKGLPSSIEKTISKAKGQPREPQVYTLPPSQEEMTKNQVSLTCLVKGFYPSDIAVEWESNGQPENNYKTTPPVLDSDGSFFLYSRLTVDKSRWQEGNVFSCSVMHEALHNHYTQKSLSLSLGK

SEQ ID NO: 22 - protein, 107 aa, synthetic construct [sequence omitted]

SEQ ID NO: 23 - DNA, 342 bp, synthetic construct
  source 1..342: mol_type = other DNA
gaggtgcagctggtgcagagcggagcagaggtgaagaagccaggggccacagtgaagataagctgtaaggtgagcggatatagctttacagggtacagaattcactgggtgcagcaggcacccggcaaaggactggagtggatgggatatgtggacccctacgatgacaagaccgactacagccagaaaagcaagggcagagtgaccattaccgcagacacaagcaccgacacagcctacatggagctgagcagcctgagaagcgaggataccgccgtgtactactgcgccagagaaggattcgcctactgggggcaagggaccctggtgaccgtgagcagc

SEQ ID NO: 24 - DNA, 318 bp, synthetic construct
  source 1..318: mol_type = other DNA
gacattcagatgacccagagccccagcagcctgagcgccagcgtgggagacagagtgaccataacctgcacctccagcagcagcctgagatacatgcactggtaccagcagaaacccgggaaggcccccaaactgctcatctacaacaccttcgacctggccagcggcgtgcccagcagattctccggcagcggaagcggaacagacttcaccctgactatcagcagcctccaacccgaagacttcgcaacttactactgccaacagcggaccacctatccacccaccttcggccagggcaccaagctggaaatcaaa

SEQ ID NO: 25 - DNA, 369 bp, synthetic construct
  source 1..369: mol_type = other DNA
caggtccaactccaagagagcggccccggcctcgtcaaacccagccaaacactctccctcacctgcacagtcagcggctacgccgtcacaggagactacgcctggagctggatcagacaaccccccggcaaaagactggagtggatcggctatatcagcagcagcgccggcaccaactacaaccccagcctgaaaagcagagtgacaataagcgtggacacttctaagaaccagttcagcctcaaactgagctccgtgaccgccgcagacaccgccgtgtactactgcgcccgagacctctactacggcggaagaaaccagtggtacttcgatgtgtggggccaaggcaccctggtgaccgtgagcagc

SEQ ID NO: 26 - DNA, 318 bp, synthetic construct
  source 1..318: mol_type = other DNA
gacattcagatgacccagagccccagcagcctgagcgccagcgtgggagacagagtgaccataacctgcagcgccacatccagcataatatatatgcactggtatcagcaaaagcccggcaaggcccccaaactgctcatctacgacaccagcaagctgcccagcggcgtgcctagccgcttctccggaagcggctccggaaccgacttcaccctcactatcagcagcctgcaacccgaagacttcgccacctactactgccaccaaagaagctccttccccttcacattcggcggtggcaccaaagtggagatcaag

SEQ ID NO: 27 - protein, 224 aa, synthetic construct
PPCPPCPAPEFLGGPSVFLFPPKPKDTLMISRTPEVTCVVVDVSQEDPEVQFNWYVDGVEVHNAKTKPREEQFNSTYRVVSVLTVLHQDWLNGKEYKCKVSNKGLPSSIEKTISKAKGQPREPQVYTLPPSQEEMTKNQVSLTCLVKGFYPSDIAVEWESNGQPENNYKTTPPVLDSDGSFFLYSRLTVDKSRWQEGNVFSCSVMHEALHNHYTQKSLSLSLGK

SEQ ID NO: 28 - protein, 224 aa, synthetic construct
PPCPSCPAPEFLGGPSVFLFPPKPKDTLMISRTPEVTCVVVDVSQEDPEVQFNWYVDGVEVHNAKTKPREEQFNSTYRVVSVLTVLHQDWLNGKEYKCKVSNKGLPSSIEKTISKAKGQPREPQVYTLPPSQEEMTKNQVSLTCLVKGFYPSDIAVEWESNGQPENNYKTTPPVLDSDGSFFLYSRLTVDKSRWQEGNVFSCSVMHEALHNHYTQKSLSLSLGK

SEQ ID NO: 29 - protein, 327 aa, synthetic construct
ASTKGPSVFPLAPCSRSTSESTAALGCLVKDYFPEPVTVSWNSGALTSGVHTFPAVLQSSGLYSLSSVVTVPSSSLGTKTYTCNVDHKPSNTKVDKRVESKYGPPCPSCPAPEFLGGPSVFLFPPKPKDTLMISRTPEVTCVVVDVSQEDPEVQFNWYVDGVEVHNAKTKPREEQFNSTYRVVSVLTVLHQDWLNGKEYKCKVSNKGLPSSIEKTISKAKGQPREPQVYTLPPSQEEMTKNQVSLTCLVKGFYPSDIAVEWESNGQPENNYKTTPPVLDSDGSFFLYSRLTVDKSRWQEGNVFSCSVMHEALHNHYTQKSLSLSLGK

SEQ ID NO: 30 - protein, 183 aa, synthetic construct
MERVQPLEENVGNAARPRFERNKLLLVASVIQGLGLLLCFTYICLHFSALQVSHRYPRIQSIKVQFTEYKKEKGFILTSQKEDEIMKVQNNSVIINCDGFYLISLKGYFSQEVNISLHYQKDEEPLFQLKKVRSVNSLMVASLTYKDKVYLNVTTDNTSLDDFHVNGGELILIHQNPGEFCVL